European Patent Application EP 4 349 363 A2, published April 10, 2024. Title: DOSING REGIMENS. Applicant: APELLIS PHARMACEUTICALS, INC. Application EP EP23209532.3, filed October 7, 2016. The sequence listing filed with the application follows.

SEQUENCE LISTING (76 sequences)

SEQ ID NO: 1 - protein, 13 aa, synthetic construct
  DISULFID 2..12: note = Intrachain
ICVVQDWGHHRCT

SEQ ID NO: 2 - protein, 42 aa, synthetic construct
  REGION 1..42: note = Description of Artificial Sequence: Synthetic polypeptide
  REGION 1..19: note = misc_feature - This region may encompass 2 to 19 residues, wherein some residues may be absent
  MOD_RES 22: note = Trp or an analog of Trp
  REGION 24..42: note = misc_feature - This region may encompass 2 to 19 residues, wherein some residues may be absent
  VARIANT 1..19: note = Any independently selected amino acid or amino acid analog
  VARIANT 24..42: note = Any independently selected amino acid or amino acid analog
XXXXXXXXXXXXXXXXXXXQDWGXXXXXXXXXXXXXXXXXXX

SEQ ID NO: 3 - protein, 5 aa, synthetic construct
  REGION 1..5: note = Description of Artificial Sequence: Synthetic peptide
  MOD_RES 1: note = Trp or an analog of Trp
  MOD_RES 4: note = Trp or an analog of Trp
WQDWG

SEQ ID NO: 4 - protein, 6 aa, synthetic construct
  REGION 1..6: note = Description of Artificial Sequence: Synthetic peptide
  MOD_RES 1: note = Trp or an analog of Trp
  MOD_RES 4: note = Trp or an analog of Trp
  VARIANT 6: note = His, Ala, analogs of Ala, Phe or Trp
WQDWGX

SEQ ID NO: 5 - protein, 13 aa, synthetic construct
  REGION 1..13: note = Description of Artificial Sequence: Synthetic peptide
  MOD_RES 4: note = Trp or analog of Trp
  MOD_RES 7: note = Trp or analog of Trp
  VARIANT 1..3: note = Any independently selected amino acid or amino acid analog
  VARIANT 9..13: note = Any independently selected amino acid or amino acid analog
XXXWQDWGXXXXX

SEQ ID NO: 6 - protein, 16 aa, synthetic construct
  REGION 1..16: note = Description of Artificial Sequence: Synthetic peptide
  REGION 1..2: note = misc_feature - This region may encompass 1 to 2 residues, wherein some positions may be absent
  MOD_RES 5: note = Independently selected from Trp or analogs of Trp
  MOD_RES 8: note = Independently selected from Trp or analogs of Trp
  REGION 14..16: note = misc_feature - This region may encompass 1 to 3 residues, wherein some positions may be absent
  VARIANT 1..2: note = Ile, Val, Leu, B1-Ile, B1-Val, B1-Leu or a dipeptide comprising Gly-Ile or B1-Gly-Ile, wherein B1 represents a first blocking moiety
  DISULFID 3..13: note = Intrachain
  VARIANT 10: note = His, Ala or an analog of Ala, Phe, Trp or an analog of Trp
  VARIANT 14..16: note = L-Thr, D-Thr, Ile, Val, Gly, a dipeptide selected from Thr-Ala or Thr-Asn, or a tripeptide comprising Thr-Ala-Asn, wherein a c-term-OH of any of the L-Thr, D-Thr, Ile, Val, Gly, Ala or Asn is optionally replaced by a second blocking moiety
XXCVWQDWGXHRCXXX

SEQ ID NO: 7 - protein, 16 aa, synthetic construct
  REGION 1..16: note = Description of Artificial Sequence: Synthetic peptide
  REGION 1..2: note = misc_feature - This region may encompass 1 to 2 residues, wherein some positions may be absent
  REGION 1..16: note = MISC_FEATURE - see specification as filed for detailed description of substitutions and preferred embodiments
  MOD_RES 5: note = Independently selected from Trp or analogs of Trp
  MOD_RES 8: note = Independently selected from Trp or analogs of Trp
  REGION 14..16: note = misc_feature - This region may encompass 1 to 3 residues, wherein some positions may be absent
  VARIANT 1..2: note = Ile, Val, Leu, Ac-Ile, Ac-Val, Ac-Leu or a dipeptide comprising Gly-Ile or Ac-Gly-Ile
  DISULFID 3..13: note = Intrachain
  VARIANT 10: note = His, Ala or an analog of Ala, Phe, Trp or an analog of Trp
  VARIANT 14..16: note = L-Thr, D-Thr, Ile, Val, Gly, a dipeptide selected from Thr-Ala or Thr-Asn, or a tripeptide comprising Thr-Ala-Asn, wherein a c-term-OH of any of L-Thr, D-Thr, Ile, Val, Gly, Ala, or Asn is optionally replaced by -NH2
XXCVWQDWGXHRCXXX

SEQ ID NO: 8 - protein, 13 aa, synthetic construct
  REGION 1..13: note = Description of Artificial Sequence: Synthetic peptide
  MOD_RES 1: note = N-term H
  MOD_RES 13: note = C-term CONH2
ICVVQDWGHHRCT

SEQ ID NO: 9 - protein, 13 aa, synthetic construct
  REGION 1..13: note = Description of Artificial Sequence: Synthetic peptide
  MOD_RES 1: note = N-term Ac
  MOD_RES 13: note = C-term CONH2
ICVVQDWGHHRCT

SEQ ID NO: 10 - protein, 13 aa, synthetic construct
  REGION 1..13: note = Description of Artificial Sequence: Synthetic peptide
  MOD_RES 1: note = N-term Ac
  MOD_RES 13: note = C-term CONH2
ICVYQDWGAHRCT

SEQ ID NO: 11 - protein, 13 aa, synthetic construct
  REGION 1..13: note = Description of Artificial Sequence: Synthetic peptide
  MOD_RES 1: note = N-term Ac
  MOD_RES 13: note = C-term COOH
ICVWQDWGAHRCT

SEQ ID NO: 12 - protein, 13 aa, synthetic construct
  REGION 1..13: note = Description of Artificial Sequence: Synthetic peptide
  SITE 1: note = MISC_FEATURE - N-term Ac
  SITE 13: note = MISC_FEATURE - C-term CONH2
ICVWQDWGAHRCT

SEQ ID NO: 13 - protein, 13 aa, synthetic construct
  REGION 1..13: note = Description of Artificial Sequence: Synthetic peptide
  MOD_RES 1: note = N-term Ac
  MOD_RES 13: note = d-Thr
  MOD_RES 13: note = C-term COOH
ICVWQDWGAHRCT

SEQ ID NO: 14 - protein, 13 aa, synthetic construct
  REGION 1..13: note = Description of Artificial Sequence: Synthetic peptide
  MOD_RES 1: note = N-term Ac
  MOD_RES 4: note = 2-Nal
  MOD_RES 13: note = C-term CONH2
ICVAQDWGAHRCT

SEQ ID NO: 15 - protein, 13 aa, synthetic construct
  REGION 1..13: note = Description of Artificial Sequence: Synthetic peptide
  MOD_RES 1: note = N-term Ac
  MOD_RES 4: note = 2-Nal
  MOD_RES 13: note = C-term COOH
ICVAQDWGAHRCT

SEQ ID NO: 16 - protein, 13 aa, synthetic construct
  REGION 1..13: note = Description of Artificial Sequence: Synthetic peptide
  MOD_RES 1: note = N-term Ac
  MOD_RES 4: note = 1-Nal
  MOD_RES 13: note = C-term COOH
ICVAQDWGAHRCT

SEQ ID NO: 17 - protein, 13 aa, synthetic construct
  REGION 1..13: note = Description of Artificial Sequence: Synthetic peptide
  MOD_RES 1: note = N-term Ac
  MOD_RES 4: note = 2-Igl
  MOD_RES 13: note = C-term CONH2
ICVGQDWGAHRCT

SEQ ID NO: 18 - protein, 13 aa, synthetic construct
  REGION 1..13: note = Description of Artificial Sequence: Synthetic peptide
  MOD_RES 1: note = N-term Ac
  MOD_RES 4: note = 2-Igl
  MOD_RES 13: note = C-term COOH
ICVGQDWGAHRCT

SEQ ID NO: 19 - protein, 13 aa, synthetic construct
  REGION 1..13: note = Description of Artificial Sequence: Synthetic peptide
  MOD_RES 1: note = N-term Ac
  MOD_RES 4: note = Dht
  MOD_RES 13: note = C-term COOH
ICVWQDWGAHRCT

SEQ ID NO: 20 - protein, 13 aa, synthetic construct
  REGION 1..13: note = Description of Artificial Sequence: Synthetic peptide
  MOD_RES 1: note = N-term Ac
  MOD_RES 4: note = Bpa
  MOD_RES 13: note = C-term COOH
ICVFQDWGAHRCT

SEQ ID NO: 21 - protein, 13 aa, synthetic construct
  REGION 1..13: note = Description of Artificial Sequence: Synthetic peptide
  MOD_RES 1: note = N-term Ac
  MOD_RES 4: note = Bpa
  MOD_RES 13: note = C-term CONH2
ICVFQDWGAHRCT

SEQ ID NO: 22 - protein, 13 aa, synthetic construct
  REGION 1..13: note = Description of Artificial Sequence: Synthetic peptide
  MOD_RES 1: note = N-term Ac
  SITE 4: note = Other - BTA
  MOD_RES 13: note = C-term COOH
ICVXQDWGAHRCT

SEQ ID NO: 23 - protein, 13 aa, synthetic construct
  REGION 1..13: note = Description of Artificial Sequence: Synthetic peptide
  MOD_RES 1: note = N-term Ac
  SITE 4: note = Other - Bta
  MOD_RES 13: note = C-term CONH2
ICVXQDWGAHRCT

SEQ ID NO: 24 - protein, 13 aa, synthetic construct
  REGION 1..13: note = Description of Artificial Sequence: Synthetic peptide
  MOD_RES 1: note = N-term Ac
  SITE 9: note = Other - 2-Abu
  MOD_RES 13: note = C-term CONH2
ICVWQDWGXHRCT

SEQ ID NO: 25 - protein, 16 aa, synthetic construct
  REGION 1..16: note = Description of Artificial Sequence: Synthetic peptide
  MOD_RES 1: note = N-term H
  MOD_RES 16: note = C-term COOH
GICVWQDWGAHRCTAN

SEQ ID NO: 26 - protein, 13 aa, synthetic construct
  REGION 1..13: note = Description of Artificial Sequence: Synthetic peptide
  MOD_RES 1: note = N-term Ac
  MOD_RES 4: note = 5f-Trp
  MOD_RES 13: note = C-term CONH2
ICVWQDWGAHRCT

SEQ ID NO: 27 - protein, 13 aa, synthetic construct
  REGION 1..13: note = Description of Artificial Sequence: Synthetic peptide
  MOD_RES 1: note = N-term Ac
  MOD_RES 4: note = 5-methyl-Trp
  MOD_RES 13: note = C-term CONH2
ICVWQDWGAHRCT

SEQ ID NO: 28 - protein, 13 aa, synthetic construct
  REGION 1..13: note = Description of Artificial Sequence: Synthetic peptide
  MOD_RES 1: note = N-term Ac
  MOD_RES 4: note = 1-methyl-Trp
  MOD_RES 13: note = C-term CONH2
ICVWQDWGAHRCT

SEQ ID NO: 29 - protein, 13 aa, synthetic construct
  REGION 1..13: note = Description of Artificial Sequence: Synthetic peptide
  MOD_RES 1: note = N-term Ac
  MOD_RES 7: note = 5f-Trp
  MOD_RES 13: note = C-term CONH2
ICVWQDWGAHRCT

SEQ ID NO: 30 - protein, 13 aa, synthetic construct
  REGION 1..13: note = Description of Artificial Sequence: Synthetic peptide
  MOD_RES 1: note = N-term Ac
  MOD_RES 4: note = 5f-Trp
  MOD_RES 7: note = 5f-Trp
  MOD_RES 13: note = C-term CONH2
ICVWQDWGAHRCT

SEQ ID NO: 31 - protein, 13 aa, synthetic construct
  REGION 1..13: note = Description of Artificial Sequence: Synthetic peptide
  MOD_RES 1: note = N-term Ac
  MOD_RES 4: note = 5-methyl-Trp
  MOD_RES 7: note = 5f-Trp
  MOD_RES 13: note = C-term CONH2
ICVWQDWGAHRCT

SEQ ID NO: 32 - protein, 13 aa, synthetic construct
  REGION 1..13: note = Description of Artificial Sequence: Synthetic peptide
  MOD_RES 1: note = N-term Ac
  MOD_RES 4: note = 1-methyl-Trp
  MOD_RES 7: note = 5f-Trp
  MOD_RES 13: note = C-term CONH2
ICVWQDWGAHRCT

SEQ ID NO: 33 - protein, 15 aa, synthetic construct
  REGION 1..15: note = Description of Artificial Sequence: Synthetic peptide
  MOD_RES 1: note = N-term H
  MOD_RES 5: note = 6f-Trp
  MOD_RES 8: note = 6f-Trp
  MOD_RES 15: note = C-term COOH
GICVWQDWGAHRCTN

SEQ ID NO: 34 - protein, 13 aa, synthetic construct
  REGION 1..13: note = Description of Artificial Sequence: Synthetic peptide
  MOD_RES 1: note = N-term Ac
  MOD_RES 4: note = 1-formyl-Trp
  MOD_RES 13: note = C-term CONH2
ICVWQDWGAHRCT

SEQ ID NO: 35 - protein, 13 aa, synthetic construct
  REGION 1..13: note = Description of Artificial Sequence: Synthetic peptide
  MOD_RES 1: note = N-term Ac
  MOD_RES 4: note = 1-methoxy-Trp
  MOD_RES 13: note = C-term CONH2
ICVWQDWGAHRCT

SEQ ID NO: 36 - protein, 15 aa, synthetic construct
  REGION 1..15: note = Description of Artificial Sequence: Synthetic peptide
  MOD_RES 1: note = N-term H
  MOD_RES 5: note = 5f-Trp
  MOD_RES 8: note = 5f-Trp
  MOD_RES 15: note = C-term COOH
GICVWQDWGAHRCTN

SEQ ID NO: 37 - protein, 13 aa, synthetic construct
  REGION 1..13: note = Description of Artificial Sequence: Synthetic peptide
  DISULFID 2..12: note = Intrachain
  MOD_RES 4: note = (1Me)Trp
ICVWQDWGAHRCT

SEQ ID NO: 38 - protein, 13 aa, synthetic construct
  REGION 1..13: note = Description of Artificial Sequence: Synthetic peptide
  MOD_RES 1: note = N-term Maleimide-(CH2)5-C(=O)
  DISULFID 2..12: note = Intrachain
  MOD_RES 4: note = (1Me)Trp
  MOD_RES 13: note = C-term NH2
ICVWQDWGAHRCT

SEQ ID NO: 39 - protein, 13 aa, synthetic construct
  REGION 1..13: note = Description of Artificial Sequence: Synthetic peptide
  MOD_RES 1: note = N-term Ac
  DISULFID 2..12: note = Intrachain
  MOD_RES 4: note = (1Me)Trp
  MOD_RES 13: note = C-term (C=O)-(CH2)5-maleimide
ICVWQDWGAHRCT

SEQ ID NO: 40 - protein, 13 aa, synthetic construct
  REGION 1..13: note = Description of Artificial Sequence: Synthetic peptide
  MOD_RES 1: note = N-term Maleimide-(CH2)2-C(=O)-NH-CH2CH2OCH2CH2O CH2CH2C(=O)
  DISULFID 2..12: note = Intrachain
  MOD_RES 4: note = (1Me)Trp
  MOD_RES 13: note = C-term NH2
ICVWQDWGAHRCT

SEQ ID NO: 41 - protein, 13 aa, synthetic construct
  REGION 1..13: note = Description of Artificial Sequence: Synthetic peptide
  MOD_RES 1: note = N-term Maleimide-(CH2)2-C(=O)-NH-CH2CH2OCH2CH2C(=O)
  DISULFID 2..12: note = Intrachain
  MOD_RES 4: note = (1Me)Trp
  MOD_RES 13: note = C-term NH2
ICVWQDWGAHRCT

SEQ ID NO: 42 - protein, 13 aa, synthetic construct
  REGION 1..13: note = Description of Artificial Sequence: Synthetic peptide
  MOD_RES 1: note = N-term Maleimide-(CH2)3-C(=O)-NH-CH2CH2OCH2CH2 OCH2C(=O)
  DISULFID 2..12: note = Intrachain
  MOD_RES 4: note = (1Me)Trp
  MOD_RES 13: note = C-term NH2
ICVWQDWGAHRCT

SEQ ID NO: 43 - protein, 13 aa, synthetic construct
  REGION 1..13: note = Description of Artificial Sequence: Synthetic peptide
  MOD_RES 1: note = N-term Maleimide-(CH2)5-C(=O)-NH-CH2CH2OCH2CH2 OCH2C(=O)
  DISULFID 2..12: note = Intrachain
  MOD_RES 4: note = (1Me)Trp
  MOD_RES 13: note = C-term NH2
ICVWQDWGAHRCT

SEQ ID NO: 44 - protein, 13 aa, synthetic construct
  REGION 1..13: note = Description of Artificial Sequence: Synthetic peptide
  MOD_RES 1: note = N-term Maleimide-(CH2)4-C(=O)-NH-CH2CH2OCH2CH2 OCH2CH2C(=O)
  DISULFID 2..12: note = Intrachain
  MOD_RES 4: note = (1Me)Trp
  MOD_RES 13: note = C-term NH2
ICVWQDWGAHRCT

SEQ ID NO: 45 - protein, 13 aa, synthetic construct
  REGION 1..13: note = Description of Artificial Sequence: Synthetic peptide
  MOD_RES 1: note = N-term Maleimide-(CH2)2-C(=O)-NH-CH2CH2OCH2CH2 OCH2CH2C(=O)
  DISULFID 2..12: note = Intrachain
  MOD_RES 4: note = (1Me)Trp
  MOD_RES 13: note = C-term NH2
ICVWQDWGAHRCT

SEQ ID NO: 46 - protein, 13 aa, synthetic construct
  REGION 1..13: note = Description of Artificial Sequence: Synthetic peptide
  MOD_RES 1: note = N-term Maleimide-(CH2)5-C(=O)-NH-CH2CH2OCH2CH2 OCH2C(=O)
  DISULFID 2..12: note = Intrachain
  MOD_RES 4: note = (1Me)Trp
  MOD_RES 13: note = C-term NH2
ICVWQDWGAHRCT

SEQ ID NO: 47 - protein, 14 aa, synthetic construct
  REGION 1..14: note = Description of Artificial Sequence: Synthetic peptide
  MOD_RES 1: note = N-term Ac
  DISULFID 2..12: note = Intrachain
  MOD_RES 4: note = (1Me)Trp
  MOD_RES 14: note = C-term NH2
ICVWQDWGAHRCTK

SEQ ID NO: 48 - protein, 19 aa, synthetic construct
  REGION 1..19: note = Description of Artificial Sequence: Synthetic peptide
  MOD_RES 1: note = N-term Ac
  DISULFID 2..12: note = Intrachain
  MOD_RES 4: note = (1Me)Trp
  MOD_RES 19: note = C-term NH2
ICVWQDWGAHRCTGGGGGK

SEQ ID NO: 49 - protein, 13 aa, synthetic construct
  REGION 1..13: note = Description of Artificial Sequence: Synthetic peptide
  MOD_RES 1: note = N-term NH2(CH2)5C(=O)
  MOD_RES 4: note = (1Me)Trp
  MOD_RES 13: note = C-term NH2
ICVWQDWGAHRCT

SEQ ID NO: 50 - protein, 13 aa, synthetic construct
  REGION 1..13: note = Description of Artificial Sequence: Synthetic peptide
  MOD_RES 1: note = N-term NH2(CH2CH2O)2CH2C(=O)
  MOD_RES 4: note = (1Me)Trp
  MOD_RES 13: note = C-term NH2
ICVWQDWGAHRCT

SEQ ID NO: 51 - protein, 14 aa, synthetic construct
  REGION 1..14: note = Description of Artificial Sequence: Synthetic peptide
  MOD_RES 1: note = N-term Ac
  DISULFID 2..12: note = Intrachain
  MOD_RES 4: note = (1Me)Trp
  MOD_RES 14: note = NH-CH2CH2OCH2CH2OCH2-C(=O)-Lys
  MOD_RES 14: note = C-term NH2
ICVWQDWGAHRCTK

SEQ ID NO: 52 - protein, 14 aa, synthetic construct
  REGION 1..14: note = Description of Artificial Sequence: Synthetic peptide
  MOD_RES 1: note = N-term Ac
  DISULFID 2..12: note = Intrachain
  MOD_RES 4: note = (1Me)Trp
  MOD_RES 14: note = Lys-(C(=O)-(CH2)5-Mal)
  MOD_RES 14: note = C-term NH2
ICVWQDWGAHRCTK

SEQ ID NO: 53 - protein, 19 aa, synthetic construct
  REGION 1..19: note = Description of Artificial Sequence: Synthetic peptide
  MOD_RES 1: note = N-term Ac
  DISULFID 2..12: note = Intrachain
  MOD_RES 4: note = (1Me)Trp
  MOD_RES 19: note = Lys-(C(=O)-(CH2)5-Mal)
  MOD_RES 19: note = C-term NH2
ICVWQDWGAHRCTGGGGGK

SEQ ID NO: 54 - protein, 13 aa, synthetic construct
  REGION 1..13: note = Description of Artificial Sequence: Synthetic peptide
  MOD_RES 1: note = N-term Mal-(CH2)5-(C(=O)-NH(CH2)5C(=O)
  MOD_RES 4: note = (1Me)Trp
  MOD_RES 13: note = C-term NH2
ICVWQDWGAHRCT

SEQ ID NO: 55 - protein, 13 aa, synthetic construct
  REGION 1..13: note = Description of Artificial Sequence: Synthetic peptide
  MOD_RES 1: note = N-term Mal-(CH2)5-(C(=O)NH(CH2CH2O)2CH2C(=O)
  MOD_RES 4: note = (1Me)Trp
  MOD_RES 13: note = C-term NH2
ICVWQDWGAHRCT

SEQ ID NO: 56 - protein, 14 aa, synthetic construct
  REGION 1..14: note = Description of Artificial Sequence: Synthetic peptide
  MOD_RES 1: note = N-term Ac
  DISULFID 2..12: note = Intrachain
  MOD_RES 4: note = (1Me)Trp
  MOD_RES 14: note = NH-CH2CH2OCH2CH2OCH2-C(=O)-Lys-(C(=O)-(CH2)5-Mal)
  MOD_RES 14: note = C-term NH2
ICVWQDWGAHRCTK

SEQ ID NO: 57 - protein, 14 aa, synthetic construct
  REGION 1..14: note = Description of Artificial Sequence: Synthetic peptide
  MOD_RES 1: note = N-term Ac
  DISULFID 2..12: note = Intrachain
  MOD_RES 4: note = (1Me)Trp
  MOD_RES 14: note = Lys-C(=O)-CH2(OCH2CH2)2NH(C(=O)-(CH2)5-Mal)
  MOD_RES 14: note = C-term NH2
ICVWQDWGAHRCTK

SEQ ID NO: 58 - protein, 13 aa, synthetic construct
  REGION 1..13: note = Description of Artificial Sequence: Synthetic peptide
  MOD_RES 1: note = N-term (CH2CH2O)nC(=O)
  REGION 1..13: note = MISC_FEATURE - see specification as filed for detailed description of substitutions and preferred embodiments
  MOD_RES 4: note = (1Me)Trp
  MOD_RES 13: note = C-term NH2
ICVWQDWGAHRCT

SEQ ID NO: 59 - protein, 14 aa, synthetic construct
  REGION 1..14: note = Description of Artificial Sequence: Synthetic peptide
  MOD_RES 1: note = N-term Ac
  REGION 1..14: note = MISC_FEATURE - see specification as filed for detailed description of substitutions and preferred embodiments
  DISULFID 2..12: note = Intrachain
  MOD_RES 4: note = (1Me)Trp
  MOD_RES 14: note = NH-CH2CH2OCH2CH2OCH2-C(=O)-Lys-C(=O)-(CH2CH2O)n
  MOD_RES 14: note = C-term NH2
ICVWQDWGAHRCTK

SEQ ID NO: 60 - protein, 14 aa, synthetic construct
  REGION 1..14: note = Description of Artificial Sequence: Synthetic peptide
  MOD_RES 1: note = N-term Ac
  REGION 1..14: note = MISC_FEATURE - see specification as filed for detailed description of substitutions and preferred embodiments
  DISULFID 2..12: note = Intrachain
  MOD_RES 4: note = (1Me)Trp
  MOD_RES 14: note = Lys-C(=O)-(CH2CH2O)n
  MOD_RES 14: note = C-term NH2
ICVWQDWGAHRCTK

SEQ ID NO: 61 - protein, 19 aa, synthetic construct
  REGION 1..19: note = Description of Artificial Sequence: Synthetic peptide
  MOD_RES 1: note = N-term Ac
  REGION 1..19: note = MISC_FEATURE - see specification as filed for detailed description of substitutions and preferred embodiments
  DISULFID 2..12: note = Intrachain
  MOD_RES 4: note = (1Me)Trp
  MOD_RES 19: note = Lys-C(=O)-(CH2CH2O)n
  MOD_RES 19: note = C-term NH2
ICVWQDWGAHRCTGGGGGK

SEQ ID NO: 62 - protein, 19 aa, synthetic construct
  REGION 1..19: note = Description of Artificial Sequence: Synthetic peptide
  MOD_RES 1: note = N-term Ac
  MOD_RES 1: note = (CH2CH2O)nC(=O)Lys
  REGION 1..19: note = MISC_FEATURE - see specification as filed for detailed description of substitutions and preferred embodiments
  DISULFID 8..18: note = Intrachain
  MOD_RES 10: note = (1Me)Trp
  MOD_RES 19: note = C-term NH2
KGGGGGICVWQDWGAHRCT

SEQ ID NO: 63 - protein, 14 aa, synthetic construct
  REGION 1..14: note = Description of Artificial Sequence: Synthetic peptide
  MOD_RES 1: note = N-term Ac
  MOD_RES 1: note = (CH2CH2O)nC(=O)Lys
  REGION 1..14: note = MISC_FEATURE - see specification as filed for detailed description of substitutions and preferred embodiments
  DISULFID 3..13: note = Intrachain
  MOD_RES 5: note = (1Me)Trp
  MOD_RES 14: note = C-term NH2
KICVWQDWGAHRCT

SEQ ID NO: 64 - protein, 14 aa, synthetic construct
  REGION 1..14: note = Description of Artificial Sequence: Synthetic peptide
  MOD_RES 1: note = N-term Ac
  REGION 1..14: note = MISC_FEATURE - see specification as filed for detailed description of substitutions and preferred embodiments
  DISULFID 2..12: note = Intrachain
  MOD_RES 4: note = (1Me)Trp
  MOD_RES 14: note = NH-CH2CH2OCH2CH2OCH2-C(=O)-Lys-(C(=O)-(CH2CH2O)n-R)
  MOD_RES 14: note = C-term NH2
ICVWQDWGAHRCTK

SEQ ID NO: 65 - protein, 14 aa, synthetic construct
  REGION 1..14: note = Description of Artificial Sequence: Synthetic peptide
  MOD_RES 1: note = N-term Ac
  REGION 1..14: note = MISC_FEATURE - see specification as filed for detailed description of substitutions and preferred embodiments
  DISULFID 2..12: note = Intrachain
  MOD_RES 4: note = (1Me)Trp
  MOD_RES 14: note = NH-CH2CH2OCH2CH2OCH2-C(=O)-Lys-(C(=O)-(CH2)m- (CH2CH2O)n-R)
  MOD_RES 14: note = C-term NH2
ICVWQDWGAHRCTK

SEQ ID NO: 66 - protein, 14 aa, synthetic construct
  REGION 1..14: note = Description of Artificial Sequence: Synthetic peptide
  MOD_RES 1: note = N-term Ac
  REGION 1..14: note = MISC_FEATURE - see specification as filed for detailed description of substitutions and preferred embodiments
  DISULFID 2..12: note = Intrachain
  MOD_RES 4: note = (1Me)Trp
  MOD_RES 14: note = NH-CH2CH2OCH2CH2OCH2-C(=O)-Lys-(C(=O)-(CH2)m-C(=O)- (CH2CH2O)n-R)
  MOD_RES 14: note = C-term NH2
ICVWQDWGAHRCTK

SEQ ID NO: 67 - protein, 14 aa, synthetic construct
  REGION 1..14: note = Description of Artificial Sequence: Synthetic peptide
  MOD_RES 1: note = N-term Ac
  DISULFID 2..12: note = Intrachain
  MOD_RES 4: note = (1Me)Trp
  MOD_RES 14: note = NH-CH2CH2OCH2CH2OCH2-C(=O)-Lys-(C(=O)-(CH2)m-C(=O) -(CH2)j(CH2CH2O)n-R)
  MOD_RES 14: note = C-term NH2
ICVWQDWGAHRCTK

SEQ ID NO: 68 - protein, 14 aa, synthetic construct
  REGION 1..14: note = Description of Artificial Sequence: Synthetic peptide
  MOD_RES 1: note = N-term Ac
  REGION 1..14: note = MISC_FEATURE - see specification as filed for detailed description of substitutions and preferred embodiments
  DISULFID 2..12: note = Intrachain
  MOD_RES 4: note = (1Me)Trp
  MOD_RES 14: note = AEEAc-Lys-(C(=O)-(CH2)5-Mal)
  MOD_RES 14: note = C-term NH2
ICVWQDWGAHRCTK

SEQ ID NO: 69 - protein, 6 aa, synthetic construct
  REGION 1..6: note = Description of Artificial Sequence: Synthetic 6xHis tag
HHHHHH

SEQ ID NO: 70 - protein, 4 aa, synthetic construct
  REGION 1..4: note = Description of Artificial Sequence: Synthetic peptide
  REGION 1..4: note = MISC_FEATURE - see specification as filed for detailed description of substitutions and preferred embodiments
  MOD_RES 3: note = Trp or an analog of Trp
QDWG

SEQ ID NO: 71 - protein, 15 aa, synthetic construct
  REGION 1..15: note = Description of Artificial Sequence: Synthetic peptide
  VARIANT 1: note = Any amino acid; comprises a blocking moiety
  VARIANT 2..4: note = Any independently selected amino acid or amino acid analog
  MOD_RES 5: note = Trp or analog of Trp
  MOD_RES 8: note = Trp or analog of Trp
  VARIANT 10..14: note = Any independently selected amino acid or amino acid analog
  VARIANT 15: note = Any amino acid; comprises a blocking moiety
XXXXWQDWGXXXXXX

SEQ ID NO: 72 - protein, 18 aa, synthetic construct
  REGION 1..18: note = Description of Artificial Sequence: Synthetic peptide
  VARIANT 1: note = Any amino acid; comprises a blocking moiety
  VARIANT 2..3: note = Ile, Val, Leu, B1-Ile, B1-Val, B1-Leu or a dipeptide comprising Gly-Ile or B1-Gly-Ile, wherein B1 represents a first blocking moiety
  REGION 2..3: note = misc_feature - This region may encompass 1 to 2 residues, wherein some positions may be absent
  REGION 4..14: note = misc_feature - Disulfide bond
  MOD_RES 6: note = Independently selected from Trp or analogs of Trp
  MOD_RES 9: note = Independently selected from Trp or analogs of Trp
  VARIANT 11: note = His, Ala or an analog of Ala, Phe, Trp or an analog of Trp
  VARIANT 15..17: note = L-Thr, D-Thr, Ile, Val, Gly, a dipeptide selected from Thr-Ala or Thr-Asn, or a tripeptide comprising Thr-Ala-Asn, wherein a c-term -OH of any of the L-Thr, D-Thr, Ile, Val, Gly, Ala or Asn is optionally replaced by a second blocking moiety
  REGION 15..17: note = misc_feature - This region may encompass 1 to 3 residues, wherein some positions may be absent
  VARIANT 18: note = Any amino acid; comprises a blocking moiety
XXXCVWQDWGXHRCXXXX

SEQ ID NO: 73 - skipped

SEQ ID NO: 74 - protein, 15 aa, synthetic construct
  REGION 1..15: note = Description of Artificial Sequence: Synthetic peptide
  VARIANT 1: note = Any amino acid; comprises a blocking moiety
  DISULFID 3..13: note = Intrachain
  MOD_RES 5: note = Trp(Me)
  MOD_RES 9: note = mGly
  MOD_RES 14: note = mIle
  VARIANT 15: note = Any amino acid; comprises a blocking moiety
XICVWQDWGAHRCIX

SEQ ID NO: 75 - protein, 15 aa, synthetic construct
  REGION 1..15: note = Description of Artificial Sequence: Synthetic peptide
  VARIANT 1: note = Any amino acid; comprises a blocking moiety
  DISULFID 3..13: note = Intrachain
  MOD_RES 5: note = Trp(Me)
  MOD_RES 9: note = mGly
  MOD_RES 14: note = mIle
  VARIANT 15: note = Any amino acid; comprises a blocking moiety
XICVWQDWGAHRCIX

SEQ ID NO: 76 - protein, 13 aa, synthetic construct
  REGION 1..13: note = Description of Artificial Sequence: Synthetic peptide
  DISULFID 2..12: note = Intrachain
  MOD_RES 4: note = (1Me)Trp
ICVWQDWGAHRCT